European Patent Application EP 4 732 675 A2, published April 29, 2026. Title: Stable Protease variants. Applicant: EW Nutrition GmbH. The sequence listing filed with the application follows.

SEQUENCE LISTING (5 sequences)

SEQ ID NO: 1 - protein, 552 aa, synthetic construct
  REGION 1..552: note = Kumamolisin 1 proenzyme, backbone variant (N-terminal M is lacking)
SDMEKPWKEGEEARAVLQGHARAQAPQAVDKGPVAGDERMAVTVVLRRQRAGELAAHVERQAAIAPHAREHLKREAFAASHGASLDDFAELRRFADAHGLALDRANVAAGTAVLSGPVDAINRAFGVELRHFDHPDGSYRSYLGEVTVPASIAPMIEAVLGLDTRPVARPHFRMQRRAEGGFEARSQAAAPTAYTPLDVAQAYQFPEGLDGQGQCIAIIELGGGYDEASLAQYFASLGVPAPQVVSVSVDGASNQPTGDPSGPDGEVELDIEVAGALAPGAKFAVYFAPNTDAGFLDAITTAIHDPTLKPSVVSISWGGPEDSWTSAAIAAMNRAFLDAAALGVTVLAAAGDSGSTDGEQDGLYHVDFPAASPYVLACGGTRLVASGGRIAQETVWNDGPDGGATGGGVSRIFPLPAWQEHANVPPSANPGASSGRGVPDLAGNADPATGYEVVIDGEATVIGGTSAVAPLFAALVARINQKLGKAVGYLNPTLYQLPADVFHDITEGNNDIANRAQIYQAGPGWDPCTGLGSPIGVRLLQALLPSASQPQP

SEQ ID NO: 2 - protein, 587 aa, synthetic construct
  REGION 1..587: note = Kumamolisin 1 proenzyme backbone variant with leader sequence and His tag
MNIKKFAKQATVLTFTTALLAGGATQAFASDMEKPWKEGEEARAVLQGHARAQAPQAVDKGPVAGDERMAVTVVLRRQRAGELAAHVERQAAIAPHAREHLKREAFAASHGASLDDFAELRRFADAHGLALDRANVAAGTAVLSGPVDAINRAFGVELRHFDHPDGSYRSYLGEVTVPASIAPMIEAVLGLDTRPVARPHFRMQRRAEGGFEARSQAAAPTAYTPLDVAQAYQFPEGLDGQGQCIAIIELGGGYDEASLAQYFASLGVPAPQVVSVSVDGASNQPTGDPSGPDGEVELDIEVAGALAPGAKFAVYFAPNTDAGFLDAITTAIHDPTLKPSVVSISWGGPEDSWTSAAIAAMNRAFLDAAALGVTVLAAAGDSGSTDGEQDGLYHVDFPAASPYVLACGGTRLVASGGRIAQETVWNDGPDGGATGGGVSRIFPLPAWQEHANVPPSANPGASSGRGVPDLAGNADPATGYEVVIDGEATVIGGTSAVAPLFAALVARINQKLGKAVGYLNPTLYQLPADVFHDITEGNNDIANRAQIYQAGPGWDPCTGLGSPIGVRLLQALLPSASQPQPHHHHHH

SEQ ID NO: 3 - protein, 364 aa, synthetic construct
  REGION 1..364: note = activated Kumamolisin 1, backbone variant
AAPTAYTPLDVAQAYQFPEGLDGQGQCIAIIELGGGYDEASLAQYFASLGVPAPQVVSVSVDGASNQPTGDPSGPDGEVELDIEVAGALAPGAKFAVYFAPNTDAGFLDAITTAIHDPTLKPSVVSISWGGPEDSWTSAAIAAMNRAFLDAAALGVTVLAAAGDSGSTDGEQDGLYHVDFPAASPYVLACGGTRLVASGGRIAQETVWNDGPDGGATGGGVSRIFPLPAWQEHANVPPSANPGASSGRGVPDLAGNADPATGYEVVIDGEATVIGGTSAVAPLFAALVARINQKLGKAVGYLNPTLYQLPADVFHDITEGNNDIANRAQIYQAGPGWDPCTGLGSPIGVRLLQALLPSASQPQP

SEQ ID NO: 4 - protein, 553 aa, Alicyclobacillus sendaiensis
MSDMEKPWKEGEEARAVLQGHARAQAPQAVDKGPVAGDERMAVTVVLRRQRAGELAAHVERQAAIAPHAREHLKREAFAASHGASLDDFAELRRFADAHGLALDRANVAAGTAVLSGPVDAINRAFGVELRHFDHPDGSYRSYLGEVTVPASIAPMIEAVLGLDTRPVARPHFRMQRRAEGGFEARSQAAAPTAYTPLDVAQAYQFPEGLDGQGQCIAIIELGGGYDEASLAQYFASLGVPAPQVVSVSVDGASNQPTGDPSGPDGEVELDIEVAGALAPGAKFAVYFAPNTDAGFLDAITTAIHDPTLKPSVVSISWGGPEDSWTSAAIAAMNRAFLDAAALGVTVLAAAGDSGSTDGEQDGLYHVDFPAASPYVLACGGTRLVASGGRIAQETVWNDGPDGGATGGGVSRIFPLPAWQEHANVPPSANPGASSGRGVPDLAGNADPATGYEVVIDGEATVIGGTSAVAPLFAALVARINQKLGKAVGYLNPTLYQLPADVFHDITEGNNDIANRAQIYQAGPGWDPCTGLGSPIGVRLLQALLPSASQPQP

SEQ ID NO: 5 - protein, 29 aa, synthetic construct
  REGION 1..29: note = sacB signal peptide
MNIKKFAKQATVLTFTTALLAGGATQAFA